European Patent Application EP 4 643 877 A1, published November 5, 2025. Title: 一种CD40结合分子的组合物及医药用途. Applicant: 苏州盛迪亚生物医药有限公司. The sequence listing filed with the application follows.

SEQUENCE LISTING (24 sequences)

SEQ ID NO: 1 - protein, 114 aa, Artificial Sequence
QSVRESEGGLVKPTDTLTLTCTVSGFSLSSYDMSWVRQAPGNGLEWIGAIGGAGGTYYASWAKSRSTITRNTNLNTVTLKMSSLTAADTATYFCARGWTRLDLWGQGTLVTVSS

SEQ ID NO: 2 - protein, 113 aa, Artificial Sequence
ADIVLTQTPSPVSGAVGGTVTIKCQASEDISSNLAWYQQKPGQPPKLLIFPASNLASGVSSRFKGSGSGTEFTLTISDLECADAATYYCQGGYWTSTSNFGNGFGGGTEVVVK

SEQ ID NO: 3 - protein, 5 aa, Artificial Sequence
SYDMS

SEQ ID NO: 4 - protein, 16 aa, Artificial Sequence
AIGGAGGTYYASWAKS

SEQ ID NO: 5 - protein, 7 aa, Artificial Sequence
GWTRLDL

SEQ ID NO: 6 - protein, 11 aa, Artificial Sequence
QASEDISSNLA

SEQ ID NO: 7 - protein, 7 aa, Artificial Sequence
PASNLAS

SEQ ID NO: 8 - protein, 14 aa, Artificial Sequence
QGGYWTSTSNFGNG

SEQ ID NO: 9 - protein, 112 aa, Artificial Sequence
DIQLTQSPSFLSASVGDRVTITCQASEDISSNLAWYQQKPGKPPKLLIFPASNLASGVPSRFSGSGSGTEFTLTISSLQPEDFATYYCQGGYWTSTSNFGNVFGGGTKVEIK

SEQ ID NO: 10 - protein, 112 aa, Artificial Sequence
DIQLTQSPSFLSASVGDRVTITCQASEDISSNLAWYQQKPGKPPKLLIFPASNLASGVPSRFSGSGSGTEFTLTISSLQPEDFATYYCQGGYWTSTSNFGSGFGGGTKVEIK

SEQ ID NO: 11 - protein, 112 aa, Artificial Sequence
DIQLTQSPSFLSASVGDRVTITCQASEDISSNLAWYQQKPGKPPKLLIFPASNLASGVPSRFSGSGSGTEFTLTISSLQPEDFATYYCQGGYWTSTSNFGTGFGGGTKVEIK

SEQ ID NO: 12 - protein, 112 aa, Artificial Sequence
DIQLTQSPSFLSASVGDRVTITCQASEDISSNLAWYQQKPGKPPKLLIFPASNLASGVPSRFSGSGSGTEFTLTISSLQPEDFATYYCQGGYWTSTSNFGQGFGGGTKVEIK

SEQ ID NO: 13 - protein, 115 aa, Artificial Sequence
EVQLQESGPGLVKPSDTLSLTCTVSGFSLSSYDMSWIRQPPGKGLEWIGAIGGAGGTYYASWAKSRVTISVDTSLNQVSLKLSSVTAADTAVYYCARGWTRLDLWGQGTLVTVSS

SEQ ID NO: 14 - protein, 115 aa, Artificial Sequence
QVQVQESGPGLVKPSDTLSLTCTVSGFSLSSYDMSWIRQPPGKGLEWIGAIGGAGGTYYASWAKSRVTISVDTSLNQVSLKLSSVTAADTAVYYCARGWTRLDLWGQGTLVTVSS

SEQ ID NO: 15 - protein, 14 aa, Artificial Sequence
QGGYWTSTSNFGNV

SEQ ID NO: 16 - protein, 14 aa, Artificial Sequence
QGGYWTSTSNFGSG

SEQ ID NO: 17 - protein, 14 aa, Artificial Sequence
QGGYWTSTSNFGTG

SEQ ID NO: 18 - protein, 14 aa, Artificial Sequence
QGGYWTSTSNFGQG

SEQ ID NO: 19 - protein, 14 aa, Artificial Sequence
  VARIANT 13: note = X can be N, S, T or Q
  VARIANT 14: note = X can be V or G
QGGYWTSTSNFGXX

SEQ ID NO: 20 - protein, 445 aa, Artificial Sequence
QVQVQESGPGLVKPSDTLSLTCTVSGFSLSSYDMSWIRQPPGKGLEWIGAIGGAGGTYYASWAKSRVTISVDTSLNQVSLKLSSVTAADTAVYYCARGWTRLDLWGQGTLVTVSSASTKGPSVFPLAPSSKSTSGGTAALGCLVKDYFPEPVTVSWNSGALTSGVHTFPAVLQSSGLYSLSSVVTVPSSSLGTQTYICNVNHKPSNTKVDKKVEPKSCDKTHTCPPCPAPELLGGPSVFLFPPKPKDTLMISRTPEVTCVVVDVSHEDPEVKFNWYVDGVEVHNAKTKPREEQYASTYRVVSVLTVLHQDWLNGKEYKCKVSNKALPAPIEKTISKAKGQPREPQVYTLPPSREEMTKNQVSLTCLVKGFYPSDIAVEWESNGQPENNYKTTPPVLDSDGSFFLYSKLTVDKSRWQQGNVFSCSVMHEALHNHYTQKSLSLSPGK

SEQ ID NO: 21 - protein, 219 aa, Artificial Sequence
DIQLTQSPSFLSASVGDRVTITCQASEDISSNLAWYQQKPGKPPKLLIFPASNLASGVPSRFSGSGSGTEFTLTISSLQPEDFATYYCQGGYWTSTSNFGQGFGGGTKVEIKRTVAAPSVFIFPPSDEQLKSGTASVVCLLNNFYPREAKVQWKVDNALQSGNSQESVTEQDSKDSTYSLSSTLTLSKADYEKHKVYACEVTHQGLSSPVTKSFNRGEC

SEQ ID NO: 22 - protein, 445 aa, Artificial Sequence
QVQVQESGPGLVKPSDTLSLTCTVSGFSLSSYDMSWIRQPPGKGLEWIGAIGGAGGTYYASWAKSRVTISVDTSLNQVSLKLSSVTAADTAVYYCARGWTRLDLWGQGTLVTVSSASTKGPSVFPLAPSSKSTSGGTAALGCLVKDYFPEPVTVSWNSGALTSGVHTFPAVLQSSGLYSLSSVVTVPSSSLGTQTYICNVNHKPSNTKVDKKVEPKSCDKTHTCPPCPAPEAAGGPSVFLFPPKPKDTLYITREPEVTCVVVDVSHEDPEVKFNWYVDGVEVHNAKTKPREEQYNSTYRVVSVLTVLHQDWLNGKEYKCKVSNKALPAPIEKTISKAKGQPREPQVYTLPPSREEMTKNQVSLTCLVKGFYPSDIAVEWESNGQPENNYKTTPPVLDSDGSFFLYSKLTVDKSRWQQGNVFSCSVMHEALHNHYTQKSLSLSPGK

SEQ ID NO: 23 - protein, 330 aa, Artificial Sequence
ASTKGPSVFPLAPSSKSTSGGTAALGCLVKDYFPEPVTVSWNSGALTSGVHTFPAVLQSSGLYSLSSVVTVPSSSLGTQTYICNVNHKPSNTKVDKKVEPKSCDKTHTCPPCPAPELLGGPSVFLFPPKPKDTLMISRTPEVTCVVVDVSHEDPEVKFNWYVDGVEVHNAKTKPREEQYASTYRVVSVLTVLHQDWLNGKEYKCKVSNKALPAPIEKTISKAKGQPREPQVYTLPPSREEMTKNQVSLTCLVKGFYPSDIAVEWESNGQPENNYKTTPPVLDSDGSFFLYSKLTVDKSRWQQGNVFSCSVMHEALHNHYTQKSLSLSPGK

SEQ ID NO: 24 - protein, 330 aa, Artificial Sequence
ASTKGPSVFPLAPSSKSTSGGTAALGCLVKDYFPEPVTVSWNSGALTSGVHTFPAVLQSSGLYSLSSVVTVPSSSLGTQTYICNVNHKPSNTKVDKKVEPKSCDKTHTCPPCPAPEAAGGPSVFLFPPKPKDTLYITREPEVTCVVVDVSHEDPEVKFNWYVDGVEVHNAKTKPREEQYNSTYRVVSVLTVLHQDWLNGKEYKCKVSNKALPAPIEKTISKAKGQPREPQVYTLPPSREEMTKNQVSLTCLVKGFYPSDIAVEWESNGQPENNYKTTPPVLDSDGSFFLYSKLTVDKSRWQQGNVFSCSVMHEALHNHYTQKSLSLSPGK